European Patent Application EP 4 321 629 A1, published February 14, 2024. Title: Method for multiplex multiple displacement amplification. Applicant: Seoul National University R&DB Foundation. The sequence listing filed with the application follows.

SEQUENCE LISTING (71 sequences)

SEQ ID NO: 1 - DNA, 15 bp, Artificial Sequence
  R15 sequence
acgctcttccgatct

SEQ ID NO: 2 - DNA, 29 bp, Artificial Sequence
  29-mer barcode primer
  misc_feature (27)..(29): Phosphorothiolate modification
acgctcttccgatctgccaagacnnnnnn

SEQ ID NO: 3 - DNA, 14 bp, Artificial Sequence
  14-mer barcode primer
  misc_feature (12)..(14): Phosphorothiolate modification
gactgtgtnnnnnn

SEQ ID NO: 4 - DNA, 13 bp, Artificial Sequence
  13-mer barcode primer
  misc_feature (11)..(13): Phosphorothiolate modification
actgtgtnnnnnn

SEQ ID NO: 5 - DNA, 12 bp, Artificial Sequence
  12-mer barcode primer
  misc_feature (10)..(12): Phosphorothiolate modification
ctgtgtnnnnnn

SEQ ID NO: 6 - DNA, 11 bp, Artificial Sequence
  11-mer barcode primer
  misc_feature (9)..(11): Phosphorothiolate modification
tgtgtnnnnnn

SEQ ID NO: 7 - DNA, 10 bp, Artificial Sequence
  10-mer barcode primer
  misc_feature (8)..(10): Phosphorothiolate modification
gtgtnnnnnn

SEQ ID NO: 8 - DNA, 12 bp, Artificial Sequence
  12-mer barcode primer
  misc_feature (1): 5' biotin modification
  misc_feature (10)..(12): Phosphorothiolate modification
actctgnnnnnn

SEQ ID NO: 9 - DNA, 12 bp, Artificial Sequence
  12-mer barcode primer
  misc_feature (1): 5' biotin modification
  misc_feature (10)..(12): Phosphorothiolate modification
cttccgnnnnnn

SEQ ID NO: 10 - DNA, 12 bp, Artificial Sequence
  12-mer barcode primer
  misc_feature (1): 5' biotin modification
  misc_feature (10)..(12): Phosphorothiolate modification
cgaactnnnnnn

SEQ ID NO: 11 - DNA, 12 bp, Artificial Sequence
  12-mer barcode primer
  misc_feature (1): 5' biotin modification
  misc_feature (10)..(12): Phosphorothiolate modification
cccgaannnnnn

SEQ ID NO: 12 - DNA, 12 bp, Artificial Sequence
  12-mer barcode primer
  misc_feature (1): 5' biotin modification
  misc_feature (10)..(12): Phosphorothiolate modification
cggcttnnnnnn

SEQ ID NO: 13 - DNA, 12 bp, Artificial Sequence
  12-mer barcode primer
  misc_feature (1): 5' biotin modification
  misc_feature (10)..(12): Phosphorothiolate modification
cacggcnnnnnn

SEQ ID NO: 14 - DNA, 12 bp, Artificial Sequence
  12-mer barcode primer
  misc_feature (1): 5' biotin modification
  misc_feature (10)..(12): Phosphorothiolate modification
ctagccnnnnnn

SEQ ID NO: 15 - DNA, 12 bp, Artificial Sequence
  12-mer barcode primer
  misc_feature (1): 5' biotin modification
  misc_feature (10)..(12): Phosphorothiolate modification
cgtgcannnnnn

SEQ ID NO: 16 - DNA, 12 bp, Artificial Sequence
  12-mer barcode primer
  misc_feature (1): 5' biotin modification
  misc_feature (10)..(12): Phosphorothiolate modification
ctatatnnnnnn

SEQ ID NO: 17 - DNA, 12 bp, Artificial Sequence
  12-mer barcode primer
  misc_feature (1): 5' biotin modification
  misc_feature (10)..(12): Phosphorothiolate modification
cccttgnnnnnn

SEQ ID NO: 18 - DNA, 12 bp, Artificial Sequence
  12-mer barcode primer
  misc_feature (1): 5' biotin modification
  misc_feature (10)..(12): Phosphorothiolate modification
cttagannnnnn

SEQ ID NO: 19 - DNA, 12 bp, Artificial Sequence
  12-mer barcode primer
  misc_feature (1): 5' biotin modification
  misc_feature (10)..(12): Phosphorothiolate modification
ctcattnnnnnn

SEQ ID NO: 20 - DNA, 12 bp, Artificial Sequence
  12-mer barcode primer
  misc_feature (1): 5' biotin modification
  misc_feature (10)..(12): Phosphorothiolate modification
aaacgannnnnn

SEQ ID NO: 21 - DNA, 12 bp, Artificial Sequence
  12-mer barcode primer
  misc_feature (1): 5' biotin modification
  misc_feature (10)..(12): Phosphorothiolate modification
atcaccnnnnnn

SEQ ID NO: 22 - DNA, 12 bp, Artificial Sequence
  12-mer barcode primer
  misc_feature (1): 5' biotin modification
  misc_feature (10)..(12): Phosphorothiolate modification
atccatnnnnnn

SEQ ID NO: 23 - DNA, 12 bp, Artificial Sequence
  12-mer barcode primer
  misc_feature (1): 5' biotin modification
  misc_feature (10)..(12): Phosphorothiolate modification
ccaaagnnnnnn

SEQ ID NO: 24 - DNA, 12 bp, Artificial Sequence
  12-mer barcode primer
  misc_feature (1): 5' biotin modification
  misc_feature (10)..(12): Phosphorothiolate modification
acatcgnnnnnn

SEQ ID NO: 25 - DNA, 12 bp, Artificial Sequence
  12-mer barcode primer
  misc_feature (1): 5' biotin modification
  misc_feature (10)..(12): Phosphorothiolate modification
actaacnnnnnn

SEQ ID NO: 26 - DNA, 12 bp, Artificial Sequence
  12-mer barcode primer
  misc_feature (1): 5' biotin modification
  misc_feature (10)..(12): Phosphorothiolate modification
cctgttnnnnnn

SEQ ID NO: 27 - DNA, 12 bp, Artificial Sequence
  12-mer barcode primer
  misc_feature (1): 5' biotin modification
  misc_feature (10)..(12): Phosphorothiolate modification
agctcannnnnn

SEQ ID NO: 28 - DNA, 12 bp, Artificial Sequence
  12-mer barcode primer
  misc_feature (1): 5' biotin modification
  misc_feature (10)..(12): Phosphorothiolate modification
aattgtnnnnnn

SEQ ID NO: 29 - DNA, 12 bp, Artificial Sequence
  12-mer barcode primer
  misc_feature (1): 5' biotin modification
  misc_feature (10)..(12): Phosphorothiolate modification
accagannnnnn

SEQ ID NO: 30 - DNA, 12 bp, Artificial Sequence
  12-mer barcode primer
  misc_feature (1): 5' biotin modification
  misc_feature (10)..(12): Phosphorothiolate modification
gtagttnnnnnn

SEQ ID NO: 31 - DNA, 12 bp, Artificial Sequence
  12-mer barcode primer
  misc_feature (1): 5' biotin modification
  misc_feature (10)..(12): Phosphorothiolate modification
tgaaacnnnnnn

SEQ ID NO: 32 - DNA, 12 bp, Artificial Sequence
  12-mer barcode primer
  misc_feature (1): 5' biotin modification
  misc_feature (10)..(12): Phosphorothiolate modification
ttattgnnnnnn

SEQ ID NO: 33 - DNA, 12 bp, Artificial Sequence
  12-mer barcode primer
  misc_feature (1): 5' biotin modification
  misc_feature (10)..(12): Phosphorothiolate modification
aaagctnnnnnn

SEQ ID NO: 34 - DNA, 12 bp, Artificial Sequence
  12-mer barcode primer
  misc_feature (1): 5' biotin modification
  misc_feature (10)..(12): Phosphorothiolate modification
tataagnnnnnn

SEQ ID NO: 35 - DNA, 12 bp, Artificial Sequence
  12-mer barcode primer
  misc_feature (1): 5' biotin modification
  misc_feature (10)..(12): Phosphorothiolate modification
ttacgtnnnnnn

SEQ ID NO: 36 - DNA, 12 bp, Artificial Sequence
  12-mer barcode primer
  misc_feature (1): 5' biotin modification
  misc_feature (10)..(12): Phosphorothiolate modification
aatacannnnnn

SEQ ID NO: 37 - DNA, 12 bp, Artificial Sequence
  12-mer barcode primer
  misc_feature (1): 5' biotin modification
  misc_feature (10)..(12): Phosphorothiolate modification
atttagnnnnnn

SEQ ID NO: 38 - DNA, 12 bp, Artificial Sequence
  12-mer barcode primer
  misc_feature (1): 5' biotin modification
  misc_feature (10)..(12): Phosphorothiolate modification
ttctacnnnnnn

SEQ ID NO: 39 - DNA, 12 bp, Artificial Sequence
  12-mer barcode primer
  misc_feature (1): 5' biotin modification
  misc_feature (10)..(12): Phosphorothiolate modification
aagtaannnnnn

SEQ ID NO: 40 - DNA, 12 bp, Artificial Sequence
  12-mer barcode primer
  misc_feature (1): 5' biotin modification
  misc_feature (10)..(12): Phosphorothiolate modification
tgactannnnnn

SEQ ID NO: 41 - DNA, 12 bp, Artificial Sequence
  12-mer barcode primer
  misc_feature (1): 5' biotin modification
  misc_feature (10)..(12): Phosphorothiolate modification
ttaacannnnnn

SEQ ID NO: 42 - DNA, 12 bp, Artificial Sequence
  12-mer barcode primer
  misc_feature (1): 5' biotin modification
  misc_feature (10)..(12): Phosphorothiolate modification
ttgaatnnnnnn

SEQ ID NO: 43 - DNA, 12 bp, Artificial Sequence
  12-mer barcode primer
  misc_feature (1): 5' biotin modification
  misc_feature (10)..(12): Phosphorothiolate modification
acggtannnnnn

SEQ ID NO: 44 - DNA, 12 bp, Artificial Sequence
  12-mer barcode primer
  misc_feature (1): 5' biotin modification
  misc_feature (10)..(12): Phosphorothiolate modification
tttgctnnnnnn

SEQ ID NO: 45 - DNA, 12 bp, Artificial Sequence
  12-mer barcode primer
  misc_feature (1): 5' biotin modification
  misc_feature (10)..(12): Phosphorothiolate modification
tttcaannnnnn

SEQ ID NO: 46 - DNA, 12 bp, Artificial Sequence
  12-mer barcode primer
  misc_feature (1): 5' biotin modification
  misc_feature (10)..(12): Phosphorothiolate modification
tacatannnnnn

SEQ ID NO: 47 - DNA, 12 bp, Artificial Sequence
  12-mer barcode primer
  misc_feature (1): 5' biotin modification
  misc_feature (10)..(12): Phosphorothiolate modification
tctagtnnnnnn

SEQ ID NO: 48 - DNA, 12 bp, Artificial Sequence
  12-mer barcode primer
  misc_feature (1): 5' biotin modification
  misc_feature (10)..(12): Phosphorothiolate modification
ttgtgannnnnn

SEQ ID NO: 49 - DNA, 12 bp, Artificial Sequence
  12-mer barcode primer
  misc_feature (1): 5' biotin modification
  misc_feature (10)..(12): Phosphorothiolate modification
tcatgcnnnnnn

SEQ ID NO: 50 - DNA, 12 bp, Artificial Sequence
  12-mer barcode primer
  misc_feature (1): 5' biotin modification
  misc_feature (10)..(12): Phosphorothiolate modification
taagtcnnnnnn

SEQ ID NO: 51 - DNA, 12 bp, Artificial Sequence
  12-mer barcode primer
  misc_feature (1): 5' biotin modification
  misc_feature (10)..(12): Phosphorothiolate modification
taaccgnnnnnn

SEQ ID NO: 52 - DNA, 12 bp, Artificial Sequence
  12-mer barcode primer
  misc_feature (1): 5' biotin modification
  misc_feature (10)..(12): Phosphorothiolate modification
tcagatnnnnnn

SEQ ID NO: 53 - DNA, 12 bp, Artificial Sequence
  12-mer barcode primer
  misc_feature (1): 5' biotin modification
  misc_feature (10)..(12): Phosphorothiolate modification
tcccagnnnnnn

SEQ ID NO: 54 - DNA, 12 bp, Artificial Sequence
  12-mer barcode primer
  misc_feature (1): 5' biotin modification
  misc_feature (10)..(12): Phosphorothiolate modification
tcgacgnnnnnn

SEQ ID NO: 55 - DNA, 12 bp, Artificial Sequence
  12-mer barcode primer
  misc_feature (1): 5' biotin modification
  misc_feature (10)..(12): Phosphorothiolate modification
tagagcnnnnnn

SEQ ID NO: 56 - DNA, 11 bp, Artificial Sequence
  11-mer barcode primer
  misc_feature (1): 5' biotin modification
  misc_feature (9)..(11): Phosphorothiolate modification
tagtcnnnnnn

SEQ ID NO: 57 - DNA, 11 bp, Artificial Sequence
  11-mer barcode primer
  misc_feature (1): 5' biotin modification
  misc_feature (9)..(11): Phosphorothiolate modification
agaagnnnnnn

SEQ ID NO: 58 - DNA, 11 bp, Artificial Sequence
  11-mer barcode primer
  misc_feature (1): 5' biotin modification
  misc_feature (9)..(11): Phosphorothiolate modification
accgannnnnn

SEQ ID NO: 59 - DNA, 11 bp, Artificial Sequence
  11-mer barcode primer
  misc_feature (1): 5' biotin modification
  misc_feature (9)..(11): Phosphorothiolate modification
tggctnnnnnn

SEQ ID NO: 60 - DNA, 11 bp, Artificial Sequence
  11-mer barcode primer
  misc_feature (1): 5' biotin modification
  misc_feature (9)..(11): Phosphorothiolate modification
agctannnnnn

SEQ ID NO: 61 - DNA, 11 bp, Artificial Sequence
  11-mer barcode primer
  misc_feature (1): 5' biotin modification
  misc_feature (9)..(11): Phosphorothiolate modification
gctctnnnnnn

SEQ ID NO: 62 - DNA, 11 bp, Artificial Sequence
  11-mer barcode primer
  misc_feature (1): 5' biotin modification
  misc_feature (9)..(11): Phosphorothiolate modification
gtgacnnnnnn

SEQ ID NO: 63 - DNA, 11 bp, Artificial Sequence
  11-mer barcode primer
  misc_feature (1): 5' biotin modification
  misc_feature (9)..(11): Phosphorothiolate modification
acagtnnnnnn

SEQ ID NO: 64 - DNA, 11 bp, Artificial Sequence
  11-mer barcode primer
  misc_feature (1): 5' biotin modification
  misc_feature (9)..(11): Phosphorothiolate modification
atgccnnnnnn

SEQ ID NO: 65 - DNA, 11 bp, Artificial Sequence
  11-mer barcode primer
  misc_feature (1): 5' biotin modification
  misc_feature (9)..(11): Phosphorothiolate modification
tactgnnnnnn

SEQ ID NO: 66 - DNA, 11 bp, Artificial Sequence
  11-mer barcode primer
  misc_feature (1): 5' biotin modification
  misc_feature (9)..(11): Phosphorothiolate modification
tcaagnnnnnn

SEQ ID NO: 67 - DNA, 11 bp, Artificial Sequence
  11-mer barcode primer
  misc_feature (1): 5' biotin modification
  misc_feature (9)..(11): Phosphorothiolate modification
cgttannnnnn

SEQ ID NO: 68 - DNA, 11 bp, Artificial Sequence
  11-mer barcode primer
  misc_feature (1): 5' biotin modification
  misc_feature (9)..(11): Phosphorothiolate modification
cctggnnnnnn

SEQ ID NO: 69 - DNA, 11 bp, Artificial Sequence
  11-mer barcode primer
  misc_feature (1): 5' biotin modification
  misc_feature (9)..(11): Phosphorothiolate modification
ttaccnnnnnn

SEQ ID NO: 70 - DNA, 11 bp, Artificial Sequence
  11-mer barcode primer
  misc_feature (1): 5' biotin modification
  misc_feature (9)..(11): Phosphorothiolate modification
gatgtnnnnnn

SEQ ID NO: 71 - DNA, 11 bp, Artificial Sequence
  11-mer barcode primer
  misc_feature (1): 5' biotin modification
  misc_feature (9)..(11): Phosphorothiolate modification
ctacannnnnn